European Patent Specification EP 3 942 298 B1, published May 7, 2025. Title: METHOD FOR INCREASING CELL SUSCEPTIBILITY TO COMPLEMENT-MEDIATED LYSIS. Applicant: The University of Alabama Research Foundation. The sequence listing filed with the application follows.

SEQUENCE LISTING (23 sequences)

SEQ ID NO: 1 - DNA, 25 bp, Artificial sequence
  Pig CD46 gRNA-1 primer
caccgctcatggacccctattgacg

SEQ ID NO: 2 - DNA, 25 bp, Artificial sequence
  Pig CD46 gRNA-2 primer
aaaccgtcaataggggtccatgagc

SEQ ID NO: 3 - DNA, 25 bp, Artificial sequence
  Pig CD55 gRNA-1 primer
caccggcgccatgagtcccctgccg

SEQ ID NO: 4 - DNA, 25 bp, Artificial sequence
  Pig CD55 gRNA-2 primer
aaaccggcaggggactcatggcgcc

SEQ ID NO: 5 - DNA, 25 bp, Artificial sequence
  Pig CD59 gRNA-1 primer
caccgaatccatagacggtcacgat

SEQ ID NO: 6 - DNA, 25 bp, Artificial sequence
  Pig CD59 gRNA-2 primer
aaacatcgtgaccgtctatggattc

SEQ ID NO: 7 - DNA, 25 bp, Artificial sequence
  Human CD46 gRNA-1 primer
caccggcgccgcgcatggagcctcc

SEQ ID NO: 8 - DNA, 25 bp, Artificial sequence
  Human CD46 gRNA-2 primer
aaacggaggctccatgcgcggcgcc

SEQ ID NO: 9 - DNA, 25 bp, Artificial sequence
  Human CD55 gRNA-1 primer
caccgggcgcgccatgaccgtcgcg

SEQ ID NO: 10 - DNA, 25 bp, Artificial sequence
  Human CD55 gRNA-2 primer
aaaccgcgacggtcatggcgcgccc

SEQ ID NO: 11 - DNA, 25 bp, Artificial sequence
  Human CD59 gRNA-1 primer
caccgatcacaatgggaatccaagg

SEQ ID NO: 12 - DNA, 25 bp, Artificial sequence
  Human CD59 gRNA-2 primer
aaacccttggattcccattgtgatc

SEQ ID NO: 13 - DNA, 634 bp, Artificial sequence
  Pig CD46 in PX330
ttggggttcgatttcttggctttatatatcttgtggaaggacgaaacaccgctcatggacccctattgacggttttagagctagaaatagcaagttaaaataaggctagtccgttatcaacttgaaaaagtggcaccgagtcggtgcttttttgttttagagctagaaatagcaagttaaaataaggctagtccgtttttagcgcgtgcgccaattctgcagacaaatggctctagaggtacccgttacataacttacggtaaatggcccgcctggctgaccgcccaacgacccccgcccattgacgtcaatagtaacgccaatagggactttccattgacgtcaatgggtggagtatttacggtaaactgcccacttggcagtacatcaagtgtatcatatgccaagtacgccccctattgacgtcaatgacggtaaatggcccgcctggcattgtgcccagtacatgaccttatgggactttcctacttggcagtacatctacgtattagtcatcgctattaccatggtcgaggtgagccccacgttctgcttcactctccccatctcccccccctccccacccccaattttgtatttatttattttttaattattttgtgcagcgatgggg

SEQ ID NO: 14 - DNA, 624 bp, Artificial sequence
  Pig CD55 in PX458
gcggattcgatttcttggctttatatatcttgtggaaggacgaaacaccggcgccatgagtcccctgccggttttagagctagaaatagcaagttaaaataaggctagtccgttatcaacttgaaaaagtggcaccgagtcggtgcttttttgttttagagctagaaatagcaagttaaaataaggctagtccgtttttagcgcgtgcgccaattctgcagacaaatggctctagaggtacccgttacataacttacggtaaatggcccgcctggctgaccgcccaacgacccccgcccattgacgtcaatagtaacgccaatagggactttccattgacgtcaatgggtggagtatttacggtaaactgcccacttggcagtacatcaagtgtatcatatgccaagtacgccccctattgacgtcaatgacggtaaatggcccgcctggcattgtgcccagtacatgaccttatgggactttcctacttggcagtacatctacgtattagtcatcgctattaccatggtcgaggtgagccccacgttctgcttcactctccccatctcccccccctccccacccccaattttgtatttatttattttttaattattttgtgca

SEQ ID NO: 15 - DNA, 634 bp, Artificial sequence
  Pig CD59 in PX330
cggaatccggatttcttggctttaatatcttgtggaaggacgaaacaccgaatccatagacggtcacgatgttttagagctagaaatagcaagttaaaataaggctagtccgttatcaacttgaaaaagtggcaccgagtcggtgcttttttgttttagagctagaaatagcaagttaaaataaggctagtccgtttttagcgcgtgcgccaattctgcagacaaatggctctagaggtacccgttacataacttacggtaaatggcccgcctggctgaccgcccaacgacccccgcccattgacgtcaatagtaacgccaatagggactttccattgacgtcaatgggtggagtatttacggtaaactgcccacttggcagtacatcaagtgtatcatatgccaagtacgccccctattgacgtcaatgacggtaaatggcccgcctggcattgtgcccagtacatgaccttatgggactttcctacttggcagtacatctacgtattagtcatcgctattaccatggtcgaggtgagccccacgttctgcttcactctccccatctcccccccctccccacccccaattttgtatttatttattttttaattattttgtgcagcgatggggg

SEQ ID NO: 16 - DNA, 603 bp, Artificial sequence
  Human CD46 in PX468
tcgggttcgatttcttggctttatatatcttgtggaaggacgaaacaccggcgccgcgcatggagcctccgttttagagctagaaatagcaagttaaaataaggctagtccgttatcaacttgaaaaagtggcaccgagtcggtgcttttttgttttagagctagaaatagcaagttaaaataaggctagtccgtttttagcgcgtgcgccaattctgcagacaaatggctctagaggtacccgttacataacttacggtaaatggcccgcctggctgaccgcccaacgacccccgcccattgacgtcaatagtaacgccaatagggactttccattgacgtcaatgggtggagtatttacggtaaactgcccacttggcagtacatcaagtgtatcatatgccaagtacgccccctattgacgtcaatgacggtaaatggcccgcctggcattgtgcccagtacatgaccttatgggactttcctacttggcagtacatctacgtattagtcatcgctattaccatggtcgaggtgagccccacgttctgcttcactctccccatctcccccccctccccacccccaattttgtatttattt

SEQ ID NO: 17 - DNA, 616 bp, Artificial sequence
  Human CD55 in PX330
acgtatcgatttcttggctttatatatcttgtggaaggacgaaacaccgggcgcgccatgaccgtcgcggttttagagctagaaatagcaagttaaaataaggctagtccgttatcaacttgaaaaagtggcaccgagtcggtgcttttttgttttagagctagaaatagcaagttaaaataaggctagtccgtttttagcgcgtgcgccaattctgcagacaaatggctctagaggtacccgttacataacttacggtaaatggcccgcctggctgaccgcccaacgacccccgcccattgacgtcaatagtaacgccaatagggactttccattgacgtcaatgggtggagtatttacggtaaactgcccacttggcagtacatcaagtgtatcatatgccaagtacgccccctattgacgtcaatgacggtaaatggcccgcctggcattgtgcccagtacatgaccttatgggactttcctacttggcagtacatctacgtattagtcatcgctattaccatggtcgaggtgagccccacgttctgcttcactctccccatctcccccccctccccacccccaattttgtatttatttattttttaattatt

SEQ ID NO: 18 - DNA, 619 bp, Artificial sequence
  Human CD59 in PX330
tcggttgcgatttcttggctttatatatcttgtggaaggacgaaacaccgatcacaatgggaatccaagggttttagagctagaaatagcaagttaaaataaggctagtccgttatcaacttgaaaaagtggcaccgagtcggtgcttttttgttttagagctagaaatagcaagttaaaataaggctagtccgtttttagcgcgtgcgccaattctgcagacaaatggctctagaggtacccgttacataacttacggtaaatggcccgcctggctgaccgcccaacgacccccgcccattgacgtcaatagtaacgccaatagggactttccattgacgtcaatgggtggagtatttacggtaaactgcccacttggcagtacatcaagtgtatcatatgccaagtacgccccctattgacgtcaatgacggtaaatggcccgcctggcattgtgcccagtacatgaccttatgggactttcctacttggcagtacatctacgtattagtcatcgctattaccatggtcgaggtgagccccacgttctgcttcactctccccatctcccccccctccccacccccaattttgtatttatttattttttaattatttt

SEQ ID NO: 19 - DNA, 2675 bp, Sus scrofa
ttgttgcgtctggtaagcctaccctaaaagctgtctcatgggttggcctcagatttcccgctgatttccccaaacatgacggtggcttgcgcaccgcgcaaggcacctcccgagcgcccagagaggcctcctttttcctggtgctgcgtggggattcttttgctggctttagtgttcccgctacccttattcgccttcgttgtctgtcctgatccaccgaaactgaagagtgcggtgctcacgagtgtccttcaacaacgttattatcctggggacaaaatagagtatcggtgtcgcccaggataccttccagatccatttgaaacccggaaatcttcctgtgaggcaaatggctcatggacccctattgacgaggcttgttttcgaaaatcatgtccgaaaccaacaatagaacatggtgaaatatatgcccctcaaagaaactttgagtttgaatcagaagttcacatttcgtgtattgaaggttaccatttaaaagggaaaggtattctaacttgtcaacttattggacaggacgtgttttggagtgatagaatgccacaatgtgaaagggtttactgtggacgacctccacaaataaaaaatggaaaacataccaatagctacaggaatatatttgaatataatgaattagtaacttatacttgtaatccttcaaatggaccagatgaatattcacttgttggagaaagcaaacttttttgttctgcacctggcaaatggagtagtgcccctcctcagtgtaaagtggtcaaatgtgaacgtccagaactcaaacatggagtcatagtatcgggaagtagagaaaaattttcctaccaagcagtggtgatatttggatgcctgcaaggtttttaccttaatggcagcaacgtggtgttctgtagtggtaataatacatgggagcctgagataccaaagtgtattaaaggttacaggccaacttatccaaccaagaatccagttgacaaatatccaggctatcctaatcccgattttgaaataccatcacttgacgactttgaggatttagatgccggaatcattgctcttatggctcttactgcaattgttgctgttgcagtagttttcacctgcctatacagatgtcttcgcagtgagaaggaggtggtgaaggataagaaaggggaggaggaagaggagcagaaggaggagaagaaggagaaagaggaggaaacagagaaaaaggaggagaaggagaagaagaaagagaaggagaaggagaagaaagagaagaagaaaaaagggaaaaaagaagctggtgctgtatccgctactcaaatggaaaaaccaaccagtccatcagtgcagaagcactaatttttcttccacaaacccatatatcagtttatcttttgattctgttaatatgttaagatctacagtaaattcatacagaaactatggaaaaccatatgtaggttcctcaaaaaattaaaaatagagctactatatgatccagcaattccactgtaggtatatatccaaagaaaacaaaatcaccagtggaagagataacagcacccactgtgtaatgcagcattgtttacagtaaccacaatatggaaacagcctaagtgtccagtgtcaaatgaatgggtgaagagaatgtgaggtagatatatagatacacacacacacacacacacacacacacacacctacacctatatatacattcataaatagatacagacagtggaataccattcaaccattaaaaagaaagccctgccatatgtgacaatacttatgaaacttgagcacattatggtaagtaaataagtcgtacagaaagacacaaatactctatgatctcacttataggtagaatccaaaaatccacacacagaaaaagaaatcagatttctggttgccagaggcaggggatgagggtggtgtaagaaatgggtgaaaggtgtcaaaaggtacaaagtagcaggtataagataagtactaggatatcatgtacagcatggtgactataattagtaatgctgtgttgtatacagctggctctgtatttgatggtcccccatccatatctgtggctatggagagctggttgtgctttgccacaatatataagagacttgagcattcaggattttatttgtaggggaagaggatgggaatctggaaccaatccccctcatatatcaagggatgacagctttacaagttgttagagggtaggtctttgatgttctgatcacaaggaagaataaaaaaaattttgtaactatgagaggtgatgcatattaagaatttattgtaatcatttcataatatttacattatcaagtcatgctgtataccctcaacttaaacagttttacacaggttacctccttttcttcttcactttgtcacacgttgcagagatggcaattttcacagtttatggcaaccctacaccagcaagtttattggtgccattttcgcaacaacatttactcattttgtgtctctgtgtcacattttggtaattcatgcagtatttaaattttttattatcatcattctgtttgttatggtgatctctgttcaattatatttcatgtcactgctgttattcactgaagatgcaaatgattattagtacttttagcaataaattattttttaattaa

SEQ ID NO: 20 - DNA, 21 bp, Artificial sequence
  Pig CD46 crispr target
gcatgggaagcaggaacacta

SEQ ID NO: 21 - protein, 392 aa, Homo sapiens [sequence omitted]

SEQ ID NO: 22 - protein, 378 aa, Sus scrofa
MMAFCALRKALPCRPENPFSSRCFVEILWVSLALVFLLPMPSDACDEPPKFESMRPQVLNTTYRPGDRVEYECRPGFQPMVPALPTSSVCQDDNTWSPLQEACRRKACSNLPDPLNGQVSYPNGDTLFGSKAQFTCNTGFYIIGAETVYCQVSGNVMAWSEPSPLCEKILCKPPGEIPNGKYTNSHKDVFEYNEVVTYSCLSSTGPDEFSLVGESSLFCIGKDEWSSDPPECKVVKCPYPVVPNGEIVSGFGSKFYYKAEVVFKCNAGFTLHGRDTIVCGANSTWEPEMPQCIKESTPPNTQPPTPSVSDSKPTDPPATPGPSHPGPPSPSDASPPKDAESLDGGIIAAIVVGVLAAIAVIAGGVYFFHHKYNKKRSK

SEQ ID NO: 23 - protein, 427 aa, Sus scrofa
MTVACAPRKAPPERPERPPFSWCCVGILLLALVFPLPLFAFVVCPDPPKLKSAVLTSVLQQRYYPGDKIEYRCRPGYLPDPFETRKSSCEANGSWTPIDEACFRKSCPKPTIEHGIYAPQRNFEFESEVHISCIEGYHLKGKGILTCQLIGQDVFWSDRMPQCERVYCGRPPQIKNGKHTNSYRNIFEYNELVTYTCNPSNGPDEYSLVGESKLFCSAPGKWSSAPPQCKVVKCERPELKHGVIVSGSREKFSYQAVVIFGCLQGFYLNGSNVVFCSGNNTWEPEIPKCIKGYRPTYPTKNPVDKYPGYPNPDFEIPSLDDFEDLDAGIIALMALTAIVAVAVVFTCLYRCLRSEKEVVKDKKGEEEEEQKEEKKEKEEETEKKEEKEKKKEKEKEKKEKKKKGKKEAGAVSATQMEKPTSPSVQKH